European Patent Specification EP 4 499 807 B1, published May 6, 2026. Title: ISOLATED FUSARIUM SOLANI IIa AND ITS USE FOR DYEING SUBSTRATES. Applicant: VTL GmbH. Application WO. The sequence listing filed with the application follows.

SEQUENCE LISTING (1 sequence)

SEQ ID NO: 1 - DNA, 683 bp, Neocosmospora lichenicola / Fusarium lichenicola
  source 1..683: mol_type = genomic DNA
tcgacctggcagtcgaccaccgtaagtcaaacctcatcgcgatctgcttatctcgggtcgtggaaccccgcctgggctcaggcggggtattcatcagtcatttcatgctgacaatcatctacagaccggtcacttgatctaccagtgcggtggtatcgacaagcgaaccatcgagaagttcgagaaggttggtgacatctccccgatcgcgccttgctattccgcatcgaactccccgtcgaattccctccctcgcgatacgctctgcgcacccttctcccgagtcccaaaaatttttgcggttcagccgtaattttctcttggtggggttatctaccccgccactcgggcgacgttgggcaaagccctgatccctgcacacaaaaacaccaaaccctcttggcgcgcatcatcacgtggtccacgacagacactaaccgattcaacaataggaagccgctgagctcggtaagggttccttcaagtacgcctgggtccttgacaagctcaaggccgagcgtgagcgtggtatcaccatcgacattgctctctggaagttcgagactccccgctactatgtcaccgtcattggtatgtcgctgtcgtctctcaaacatgtctcaccactaaccatcaacagacgcccccggccaccgtgacttcatcaagaacatgatcactgg